European Patent Application EP 4 686 477 A1, published February 4, 2026. Title: COMPOUNDS AND COMPOSITIONS FOR TREATING PNS INJURY AND DEGENERATIVE DISEASES. Applicant: AdRegeneer AG. The sequence listing filed with the application follows.

SEQUENCE LISTING (8 sequences)

SEQ ID NO: 1 - DNA, 21 bp, Homo sapiens
  source 1..21: mol_type = other DNA
gggaagggatggtactacagt

SEQ ID NO: 2 - DNA, 21 bp, Homo sapiens
  source 1..21: mol_type = other DNA
gtgaaagcgtactaaaggaag

SEQ ID NO: 3 - DNA, 21 bp, Homo sapiens
  source 1..21: mol_type = other DNA
ggtgggtgcaaactctacagc

SEQ ID NO: 4 - DNA, 21 bp, Homo sapiens
  source 1..21: mol_type = other DNA
gaccatcaaggtgggtgcaaa

SEQ ID NO: 5 - DNA, 1357 bp, Homo sapiens
  source 1..1357: mol_type = other DNA
atgagctcaggcaagagtgcccgctacaaccgcttctccggggggcccagcaatcttcccaccccagacgtcaccacagggaccagaatggaaacgaccttcggacccgccttttcagccgtcaccaccatcacaaaagctgacgggaccagcacctacaagcagcactgcaggacaccctcctcctccagcacccttgcctactccccgcgggacgaggaggacagcatgccccccatcagcactccccgccgctccgactccgccatctctgtccgctccctgcactcagagtccagcatgtctctgcgctccacattctcactgcccgaggaggaggaggagccggagccactggtgtttgcggagcagccctcggtgaagctgtgctgtcagctctgctgcagcgtcttcaaagaccccgtgatcaccacgtgtgggcacacgttctgtaggagatgcgccttgaagtcagagaagtgtcccgtggacaacgtcaaactgaccgtggtggtgaacaacatcgcggtggccgagcagatcggggagctcttcatccactgccggcacggctgccgggtagcgggcagcgggaagccccccatctttgaggtggacccccgagggtgccccttcaccatcaagctcagcgcccggaaggaccacgagggcagctgtgactacaggcctgtgcggtgtcccaacaaccccagctgccccccgctgctcaggatgaacctggaggcccacctcaaggagtgcgagcacatcaaatgcccccactccaagtacgggtgcacgttcatcgggaaccaggacacttacgagacccacctggagacttgccgcttcgagggcctgaaggagtttctgcagcagacggatgaccgcttccacgagatgcacgtggctctggcccagaaggaccaggagatcgccttcctgcgctccatgctgggaaagctctcggagaagatcgaccagctagagaagagcctggagctcaagtttgacgtcctggacgaaaaccagagcaagctcagcgaggacctcatggagttccggcgggacgcatccatgttaaatgacgagctgtcccacatcaacgcgcggctgaacatgggcatcctaggctcctacgaccctcagcagatcttcaagtgcaaagggacctttgtgggccaccagggccctgtgtggtgtctctgcgtctactccatgggtgacctgctcttcagtggctcctctgacaagaccatcaaggtgggtgcaaactctacagcggctctgcagactgcaccatcattgtgtgggacatccagaacctgcagaaggtgaacaccatccgggcccatga

SEQ ID NO: 6 - protein, 452 aa, Homo sapiens
MSSGKSARYNRFSGGPSNLPTPDVTTGTRMETTFGPAFSAVTTITKADGTSTYKQHCRTPSSSSTLAYSPRDEEDSMPPISTPRRSDSAISVRSLHSESSMSLRSTFSLPEEEEEPEPLVFAEQPSVKLCCQLCCSVFKDPVITTCGHTFCRRCALKSEKCPVDNVKLTVVVNNIAVAEQIGELFIHCRHGCRVAGSGKPPIFEVDPRGCPFTIKLSARKDHEGSCDYRPVRCPNNPSCPPLLRMNLEAHLKECEHIKCPHSKYGCTFIGNQDTYETHLETCRFEGLKEFLQQTDDRFHEMHVALAQKDQEIAFLRSMLGKLSEKIDQLEKSLELKFDVLDENQSKLSEDLMEFRRDASMLNDELSHINARLNMGILGSYDPQQIFKCKGTFVGHQGPVWCLCVYSMGDLLFSGSSDKTIKVWVQTLQRLCRLHHHCVGHPEPAEGEHHPGP

SEQ ID NO: 7 - DNA, 55 bp, synthetic construct
  source 1..55: mol_type = other DNA
tgggaagggatggtactacattcaagagatgtagtaccatcccttcccttttttc

SEQ ID NO: 8 - DNA, 59 bp, synthetic construct
  source 1..59: mol_type = other DNA
tcgagaaaaaagggaagggatggtactacgtctcttgaacgtagtaccatcccttccca